European Patent Application EP 4 151 749 A1, published March 22, 2023. Title: Oligonucléotide à double structure tige-boucle et utilisations dans la détection d'analytes d'intérêt. Applicant: Commissariat a l'Energie Atomique et aux Energies Alternatives. Application EP EP22195865.5, filed September 15, 2022. The sequence listing filed with the application follows.

SEQUENCE LISTING (14 sequences)

SEQ ID NO: 1 - DNA, 152 bp, synthetic construct
  source 1..152: mol_type = other DNA
cggatccaagacgcggtttatcgtgcagtacgccaacctttctcaataaaccgcgtcttggatccgtggttggtgtggttgggacatctctgagttatatctttccccccctcactgaccctccttcgggggaaagatataactcagagatg

SEQ ID NO: 2 - DNA, 162 bp, synthetic construct
  source 1..162: mol_type = other DNA
ggttggtgtggttggttttttttttcggatccaagacgcggtttatcgtgcagtacgccaacctttctcaataaaccgcgtcttggatccgtgacatctctgagttatatctttccccccctcactgaccctccttcgggggaaagatataactcagagatg

SEQ ID NO: 3 - DNA, 162 bp, synthetic construct
  source 1..162: mol_type = other DNA
cggatccaagacgcggtttatcgtgcagtacgccaacctttctcaataaaccgcgtcttggatccgtgacatctctgagttatatctttccccccctcactgaccctccttcgggggaaagatataactcagagatgttttttttttggttggtgtggttgg

SEQ ID NO: 4 - DNA, 45 bp, synthetic construct
  source 1..45: mol_type = other DNA
cggatccaagacgcggtttatcgtgcagtacgccaacctttctca

SEQ ID NO: 5 - DNA, 43 bp, synthetic construct
  source 1..43: mol_type = other DNA
catctctgagttatatctttcccccgaaggagggtcagtgagg

SEQ ID NO: 6 - DNA, 159 bp, synthetic construct
  source 1..159: mol_type = other DNA
agagcagcagaagtggcacaggtgattgtgaagaagaagagtgtgccacttctgctgctctcgtgcagtacgccaacctttctcatgcgctgcccctcttatcaacctgaagaagagcaggcagtgaggacaatcagttcttgctcttcttcaggttga

SEQ ID NO: 7 - DNA, 172 bp, synthetic construct
  source 1..172: mol_type = other DNA
cgtgcagtacgccaacctttctcatgcgctgcccctcttattttttttttagagcagcagaagtggcacaggtgattgtgaagaagaagagtgtgccacttctgctgctctttatcaacctgaagaagagcaggcagtgaggacaatcagttcttgctcttcttcaggttga

SEQ ID NO: 8 - DNA, 41 bp, synthetic construct
  source 1..41: mol_type = other DNA
agagcagcagaagtggcacaggtgattgtgaagaagaagag

SEQ ID NO: 9 - DNA, 40 bp, synthetic construct
  source 1..40: mol_type = other DNA
tcaacctgaagaagagcaagaactgattgtcctcactgcc

SEQ ID NO: 10 - DNA, 24 bp, synthetic construct
  source 1..24: mol_type = other DNA
gaccggtatgcgacctggtatgcg

SEQ ID NO: 11 - DNA, 24 bp, synthetic construct
  source 1..24: mol_type = other DNA
cgcataccaggtcgcataccggtc

SEQ ID NO: 12 - DNA, 15 bp, synthetic construct
  source 1..15: mol_type = other DNA
ccaaccacaccaacc

SEQ ID NO: 13 - DNA, 39 bp, synthetic construct
  source 1..39: mol_type = other DNA
ccaaccacaccaaccgaccggtatgcgacctggtatgcg

SEQ ID NO: 14 - DNA, 29 bp, synthetic construct
  source 1..29: mol_type = other DNA
agtccgtggtagggcaggttggggtgact